European Patent Application EP 4 674 958 A1, published January 7, 2026. Title: MUTANT PROLYL ISOMERASE AND GLUTAMATE-BASED AMINO ACID PRODUCTION METHOD USING SAME. Applicant: CJ CheilJedang Corporation. The sequence listing filed with the application follows.

SEQUENCE LISTING (64 sequences)

SEQ ID NO: 1 - protein, 118 aa, unidentified
MEKPQIELPVGPAPEDLVISDIIVGEGAEARPGGEVEVHYVGVDLETGEEFDSSWDRGQTSQFPLNGLIAGWQEGIPGMKVGGRRQLTIPPEAAYGPEGSGHPLSGRTLVFIIDLISA

SEQ ID NO: 2 - DNA, 357 bp, unidentified
  source 1..357: mol_type = genomic DNA
atggaaaagccacagattgagctaccggtcggtccagcaccggaagatctcgtaatctctgacatcatcgttggcgaaggcgcagaagcccgcccaggcggagaagttgaggtccactatgtgggcgttgaccttgaaaccggcgaggagtttgactcttcctgggatcgtggacagaccagccagttcccactcaacggcctcattgcaggttggcaagaaggaattccaggcatgaaggtcggcggacgtcgtcagctgaccattccgccagaggctgcttacggccctgagggttccggccacccactgtctggccgtaccctggtgttcatcatcgatttgatcagcgcataa

SEQ ID NO: 3 - protein, 118 aa, synthetic construct
MEKPQIELPVGPAPEDLVISDIIVGEGAEARPGGEVEVHYVGVDLETGEEFDSSWDRGQTSQFPLNGLIAGWQEGIPGMKVGGRRQLTIPPEAAMGPEGSGHPLSGRTLVFIIDLISA

SEQ ID NO: 4 - DNA, 357 bp, synthetic construct
  source 1..357: mol_type = other DNA
atggaaaagccacagattgagctaccggtcggtccagcaccggaagatctcgtaatctctgacatcatcgttggcgaaggcgcagaagcccgcccaggcggagaagttgaggtccactatgtgggcgttgaccttgaaaccggcgaggagtttgactcttcctgggatcgtggacagaccagccagttcccactcaacggcctcattgcaggttggcaagaaggaattccaggcatgaaggtcggcggacgtcgtcagctgaccattccgccagaggctgctatgggccctgagggttccggccacccactgtctggccgtaccctggtgttcatcatcgatttgatcagcgcataa

SEQ ID NO: 5 - protein, 118 aa, synthetic construct
MEKPQIELPVGPAPEDLVISDIIVGEGAEARPGGEVEVHYVGVDLETGEEFDSSWDRGQTSQFPLNGLIAGWQEGIPGMKVGGRRQLTIPPEAASGPEGSGHPLSGRTLVFIIDLISA

SEQ ID NO: 6 - DNA, 357 bp, synthetic construct
  source 1..357: mol_type = other DNA
atggaaaagccacagattgagctaccggtcggtccagcaccggaagatctcgtaatctctgacatcatcgttggcgaaggcgcagaagcccgcccaggcggagaagttgaggtccactatgtgggcgttgaccttgaaaccggcgaggagtttgactcttcctgggatcgtggacagaccagccagttcccactcaacggcctcattgcaggttggcaagaaggaattccaggcatgaaggtcggcggacgtcgtcagctgaccattccgccagaggctgcttccggccctgagggttccggccacccactgtctggccgtaccctggtgttcatcatcgatttgatcagcgcataa

SEQ ID NO: 7 - protein, 118 aa, synthetic construct
MEKPQIELPVGPAPEDLVISDIIVGEGAEARPGGEVEVHYVGVDLETGEEFDSSWDRGQTSQFPLNGLIAGWQEGIPGMKVGGRRQLTIPPEAATGPEGSGHPLSGRTLVFIIDLISA

SEQ ID NO: 8 - DNA, 357 bp, synthetic construct
  source 1..357: mol_type = other DNA
atggaaaagccacagattgagctaccggtcggtccagcaccggaagatctcgtaatctctgacatcatcgttggcgaaggcgcagaagcccgcccaggcggagaagttgaggtccactatgtgggcgttgaccttgaaaccggcgaggagtttgactcttcctgggatcgtggacagaccagccagttcccactcaacggcctcattgcaggttggcaagaaggaattccaggcatgaaggtcggcggacgtcgtcagctgaccattccgccagaggctgctaccggccctgagggttccggccacccactgtctggccgtaccctggtgttcatcatcgatttgatcagcgcataa

SEQ ID NO: 9 - protein, 118 aa, synthetic construct
MEKPQIELPVGPAPEDLVISDIIVGEGAEARPGGEVEVHYVGVDLETGEEFDSSWDRGQTSQFPLNGLIAGWQEGIPGMKVGGRRQLTIPPEAANGPEGSGHPLSGRTLVFIIDLISA

SEQ ID NO: 10 - DNA, 357 bp, synthetic construct
  source 1..357: mol_type = other DNA
atggaaaagccacagattgagctaccggtcggtccagcaccggaagatctcgtaatctctgacatcatcgttggcgaaggcgcagaagcccgcccaggcggagaagttgaggtccactatgtgggcgttgaccttgaaaccggcgaggagtttgactcttcctgggatcgtggacagaccagccagttcccactcaacggcctcattgcaggttggcaagaaggaattccaggcatgaaggtcggcggacgtcgtcagctgaccattccgccagaggctgctaacggccctgagggttccggccacccactgtctggccgtaccctggtgttcatcatcgatttgatcagcgcataa

SEQ ID NO: 11 - protein, 118 aa, synthetic construct
MEKPQIELPVGPAPEDLVISDIIVGEGAEARPGGEVEVHYVGVDLETGEEFDSSWDRGQTSQFPLNGLIAGWQEGIPGMKVGGRRQLTIPPEAACGPEGSGHPLSGRTLVFIIDLISA

SEQ ID NO: 12 - DNA, 357 bp, synthetic construct
  source 1..357: mol_type = other DNA
atggaaaagccacagattgagctaccggtcggtccagcaccggaagatctcgtaatctctgacatcatcgttggcgaaggcgcagaagcccgcccaggcggagaagttgaggtccactatgtgggcgttgaccttgaaaccggcgaggagtttgactcttcctgggatcgtggacagaccagccagttcccactcaacggcctcattgcaggttggcaagaaggaattccaggcatgaaggtcggcggacgtcgtcagctgaccattccgccagaggctgcttgcggccctgagggttccggccacccactgtctggccgtaccctggtgttcatcatcgatttgatcagcgcataa

SEQ ID NO: 13 - protein, 118 aa, synthetic construct
MEKPQIELPVGPAPEDLVISDIIVGEGAEARPGGEVEVHYVGVDLETGEEFDSSWDRGQTSQFPLNGLIAGWQEGIPGMKVGGRRQLTIPPEAAHGPEGSGHPLSGRTLVFIIDLISA

SEQ ID NO: 14 - DNA, 357 bp, synthetic construct
  source 1..357: mol_type = other DNA
atggaaaagccacagattgagctaccggtcggtccagcaccggaagatctcgtaatctctgacatcatcgttggcgaaggcgcagaagcccgcccaggcggagaagttgaggtccactatgtgggcgttgaccttgaaaccggcgaggagtttgactcttcctgggatcgtggacagaccagccagttcccactcaacggcctcattgcaggttggcaagaaggaattccaggcatgaaggtcggcggacgtcgtcagctgaccattccgccagaggctgctcacggccctgagggttccggccacccactgtctggccgtaccctggtgttcatcatcgatttgatcagcgcataa

SEQ ID NO: 15 - protein, 118 aa, synthetic construct
MEKPQIELPVGPAPEDLVISDIIVGEGAEARPGGEVEVHYVGVDLETGEEFDSSWDRGQTSQFPLNGLIAGWQEGIPGMKVGGRRQLTIPPEAAKGPEGSGHPLSGRTLVFIIDLISA

SEQ ID NO: 16 - DNA, 357 bp, synthetic construct
  source 1..357: mol_type = other DNA
atggaaaagccacagattgagctaccggtcggtccagcaccggaagatctcgtaatctctgacatcatcgttggcgaaggcgcagaagcccgcccaggcggagaagttgaggtccactatgtgggcgttgaccttgaaaccggcgaggagtttgactcttcctgggatcgtggacagaccagccagttcccactcaacggcctcattgcaggttggcaagaaggaattccaggcatgaaggtcggcggacgtcgtcagctgaccattccgccagaggctgctaagggccctgagggttccggccacccactgtctggccgtaccctggtgttcatcatcgatttgatcagcgcataa

SEQ ID NO: 17 - protein, 118 aa, synthetic construct
MEKPQIELPVGPAPEDLVISDIIVGEGAEARPGGEVEVHYVGVDLETGEEFDSSWDRGQTSQFPLNGLIAGWQEGIPGMKVGGRRQLTIPPEAADGPEGSGHPLSGRTLVFIIDLISA

SEQ ID NO: 18 - DNA, 357 bp, synthetic construct
  source 1..357: mol_type = other DNA
atggaaaagccacagattgagctaccggtcggtccagcaccggaagatctcgtaatctctgacatcatcgttggcgaaggcgcagaagcccgcccaggcggagaagttgaggtccactatgtgggcgttgaccttgaaaccggcgaggagtttgactcttcctgggatcgtggacagaccagccagttcccactcaacggcctcattgcaggttggcaagaaggaattccaggcatgaaggtcggcggacgtcgtcagctgaccattccgccagaggctgctgatggccctgagggttccggccacccactgtctggccgtaccctggtgttcatcatcgatttgatcagcgcataa

SEQ ID NO: 19 - protein, 118 aa, synthetic construct
MEKPQIELPVGPAPEDLVISDIIVGEGAEARPGGEVEVHYVGVDLETGEEFDSSWDRGQTSQFPLNGLIAGWQEGIPGMKVGGRRQLTIPPEAAAGPEGSGHPLSGRTLVFIIDLISA

SEQ ID NO: 20 - DNA, 357 bp, synthetic construct
  source 1..357: mol_type = other DNA
atggaaaagccacagattgagctaccggtcggtccagcaccggaagatctcgtaatctctgacatcatcgttggcgaaggcgcagaagcccgcccaggcggagaagttgaggtccactatgtgggcgttgaccttgaaaccggcgaggagtttgactcttcctgggatcgtggacagaccagccagttcccactcaacggcctcattgcaggttggcaagaaggaattccaggcatgaaggtcggcggacgtcgtcagctgaccattccgccagaggctgctgcaggccctgagggttccggccacccactgtctggccgtaccctggtgttcatcatcgatttgatcagcgcataa

SEQ ID NO: 21 - protein, 118 aa, synthetic construct
MEKPQIELPVGPAPEDLVISDIIVGEGAEARPGGEVEVHYVGVDLETGEEFDSSWDRGQTSQFPLNGLIAGWQEGIPGMKVGGRRQLTIPPEAAVGPEGSGHPLSGRTLVFIIDLISA

SEQ ID NO: 22 - DNA, 357 bp, synthetic construct
  source 1..357: mol_type = other DNA
atggaaaagccacagattgagctaccggtcggtccagcaccggaagatctcgtaatctctgacatcatcgttggcgaaggcgcagaagcccgcccaggcggagaagttgaggtccactatgtgggcgttgaccttgaaaccggcgaggagtttgactcttcctgggatcgtggacagaccagccagttcccactcaacggcctcattgcaggttggcaagaaggaattccaggcatgaaggtcggcggacgtcgtcagctgaccattccgccagaggctgctgtgggccctgagggttccggccacccactgtctggccgtaccctggtgttcatcatcgatttgatcagcgcataa

SEQ ID NO: 23 - protein, 118 aa, synthetic construct
MEKPQIELPVGPAPEDLVISDIIVGEGAEARPGGEVEVHYVGVDLETGEEFDSSWDRGQTSQFPLNGLIAGWQEGIPGMKVGGRRQLTIPPEAALGPEGSGHPLSGRTLVFIIDLISA

SEQ ID NO: 24 - DNA, 357 bp, synthetic construct
  source 1..357: mol_type = other DNA
atggaaaagccacagattgagctaccggtcggtccagcaccggaagatctcgtaatctctgacatcatcgttggcgaaggcgcagaagcccgcccaggcggagaagttgaggtccactatgtgggcgttgaccttgaaaccggcgaggagtttgactcttcctgggatcgtggacagaccagccagttcccactcaacggcctcattgcaggttggcaagaaggaattccaggcatgaaggtcggcggacgtcgtcagctgaccattccgccagaggctgctctgggccctgagggttccggccacccactgtctggccgtaccctggtgttcatcatcgatttgatcagcgcataa

SEQ ID NO: 25 - protein, 118 aa, synthetic construct
MEKPQIELPVGPAPEDLVISDIIVGEGAEARPGGEVEVHYVGVDLETGEEFDSSWDRGQTSQFPLNGLIAGWQEGIPGMKVGGRRQLTIPPEAAQGPEGSGHPLSGRTLVFIIDLISA

SEQ ID NO: 26 - DNA, 357 bp, synthetic construct
  source 1..357: mol_type = other DNA
atggaaaagccacagattgagctaccggtcggtccagcaccggaagatctcgtaatctctgacatcatcgttggcgaaggcgcagaagcccgcccaggcggagaagttgaggtccactatgtgggcgttgaccttgaaaccggcgaggagtttgactcttcctgggatcgtggacagaccagccagttcccactcaacggcctcattgcaggttggcaagaaggaattccaggcatgaaggtcggcggacgtcgtcagctgaccattccgccagaggctgctcagggccctgagggttccggccacccactgtctggccgtaccctggtgttcatcatcgatttgatcagcgcataa

SEQ ID NO: 27 - protein, 118 aa, synthetic construct
MEKPQIELPVGPAPEDLVISDIIVGEGAEARPGGEVEVHYVGVDLETGEEFDSSWDRGQTSQFPLNGLIAGWQEGIPGMKVGGRRQLTIPPEAAGGPEGSGHPLSGRTLVFIIDLISA

SEQ ID NO: 28 - DNA, 357 bp, synthetic construct
  source 1..357: mol_type = other DNA
atggaaaagccacagattgagctaccggtcggtccagcaccggaagatctcgtaatctctgacatcatcgttggcgaaggcgcagaagcccgcccaggcggagaagttgaggtccactatgtgggcgttgaccttgaaaccggcgaggagtttgactcttcctgggatcgtggacagaccagccagttcccactcaacggcctcattgcaggttggcaagaaggaattccaggcatgaaggtcggcggacgtcgtcagctgaccattccgccagaggctgctggcggccctgagggttccggccacccactgtctggccgtaccctggtgttcatcatcgatttgatcagcgcataa

SEQ ID NO: 29 - protein, 118 aa, synthetic construct
MEKPQIELPVGPAPEDLVISDIIVGEGAEARPGGEVEVHYVGVDLETGEEFDSSWDRGQTSQFPLNGLIAGWQEGIPGMKVGGRRQLTIPPEAAPGPEGSGHPLSGRTLVFIIDLISA

SEQ ID NO: 30 - DNA, 357 bp, synthetic construct
  source 1..357: mol_type = other DNA
atggaaaagccacagattgagctaccggtcggtccagcaccggaagatctcgtaatctctgacatcatcgttggcgaaggcgcagaagcccgcccaggcggagaagttgaggtccactatgtgggcgttgaccttgaaaccggcgaggagtttgactcttcctgggatcgtggacagaccagccagttcccactcaacggcctcattgcaggttggcaagaaggaattccaggcatgaaggtcggcggacgtcgtcagctgaccattccgccagaggctgctccaggccctgagggttccggccacccactgtctggccgtaccctggtgttcatcatcgatttgatcagcgcataa

SEQ ID NO: 31 - protein, 118 aa, synthetic construct
MEKPQIELPVGPAPEDLVISDIIVGEGAEARPGGEVEVHYVGVDLETGEEFDSSWDRGQTSQFPLNGLIAGWQEGIPGMKVGGRRQLTIPPEAAEGPEGSGHPLSGRTLVFIIDLISA

SEQ ID NO: 32 - DNA, 357 bp, synthetic construct
  source 1..357: mol_type = other DNA
atggaaaagccacagattgagctaccggtcggtccagcaccggaagatctcgtaatctctgacatcatcgttggcgaaggcgcagaagcccgcccaggcggagaagttgaggtccactatgtgggcgttgaccttgaaaccggcgaggagtttgactcttcctgggatcgtggacagaccagccagttcccactcaacggcctcattgcaggttggcaagaaggaattccaggcatgaaggtcggcggacgtcgtcagctgaccattccgccagaggctgctgaaggccctgagggttccggccacccactgtctggccgtaccctggtgttcatcatcgatttgatcagcgcataa

SEQ ID NO: 33 - DNA, 33 bp, synthetic construct
  source 1..33: mol_type = other DNA
tcggtacccggggatccgtattgttcgcaatcg

SEQ ID NO: 34 - DNA, 25 bp, synthetic construct
  source 1..25: mol_type = other DNA
agcagcctctggcggaatggtcagc

SEQ ID NO: 35 - DNA, 35 bp, synthetic construct
  source 1..35: mol_type = other DNA
tccgccagaggctgctatgggccctgagggttccg

SEQ ID NO: 36 - DNA, 35 bp, synthetic construct
  source 1..35: mol_type = other DNA
tccgccagaggctgcttccggccctgagggttccg

SEQ ID NO: 37 - DNA, 35 bp, synthetic construct
  source 1..35: mol_type = other DNA
tccgccagaggctgctaccggccctgagggttccg

SEQ ID NO: 38 - DNA, 35 bp, synthetic construct
  source 1..35: mol_type = other DNA
tccgccagaggctgctaacggccctgagggttccg

SEQ ID NO: 39 - DNA, 35 bp, synthetic construct
  source 1..35: mol_type = other DNA
tccgccagaggctgcttgcggccctgagggttccg

SEQ ID NO: 40 - DNA, 35 bp, synthetic construct
  source 1..35: mol_type = other DNA
tccgccagaggctgctcacggccctgagggttccg

SEQ ID NO: 41 - DNA, 35 bp, synthetic construct
  source 1..35: mol_type = other DNA
tccgccagaggctgctaagggccctgagggttccg

SEQ ID NO: 42 - DNA, 35 bp, synthetic construct
  source 1..35: mol_type = other DNA
tccgccagaggctgctgatggccctgagggttccg

SEQ ID NO: 43 - DNA, 35 bp, synthetic construct
  source 1..35: mol_type = other DNA
tccgccagaggctgctgcaggccctgagggttccg

SEQ ID NO: 44 - DNA, 35 bp, synthetic construct
  source 1..35: mol_type = other DNA
tccgccagaggctgctgtgggccctgagggttccg

SEQ ID NO: 45 - DNA, 35 bp, synthetic construct
  source 1..35: mol_type = other DNA
tccgccagaggctgctctgggccctgagggttccg

SEQ ID NO: 46 - DNA, 35 bp, synthetic construct
  source 1..35: mol_type = other DNA
tccgccagaggctgctcagggccctgagggttccg

SEQ ID NO: 47 - DNA, 35 bp, synthetic construct
  source 1..35: mol_type = other DNA
tccgccagaggctgctggcggccctgagggttccg

SEQ ID NO: 48 - DNA, 35 bp, synthetic construct
  source 1..35: mol_type = other DNA
tccgccagaggctgctccaggccctgagggttccg

SEQ ID NO: 49 - DNA, 35 bp, synthetic construct
  source 1..35: mol_type = other DNA
tccgccagaggctgctgaaggccctgagggttccg

SEQ ID NO: 50 - DNA, 35 bp, synthetic construct
  source 1..35: mol_type = other DNA
tgcaggtcgactctagactgccgatcgtgtccatc

SEQ ID NO: 51 - DNA, 20 bp, synthetic construct
  source 1..20: mol_type = other DNA
tattacgccagctggcgaaa

SEQ ID NO: 52 - DNA, 20 bp, synthetic construct
  source 1..20: mol_type = other DNA
gctttacactttatgcttcc

SEQ ID NO: 53 - DNA, 36 bp, synthetic construct
  source 1..36: mol_type = other DNA
cggtacccggggatccctcgtgcggaattcgtggag

SEQ ID NO: 54 - DNA, 20 bp, synthetic construct
  source 1..20: mol_type = other DNA
atccagcagcaattcagaca

SEQ ID NO: 55 - DNA, 37 bp, synthetic construct
  source 1..37: mol_type = other DNA
ctgaattgctgctggattaaggcatcgatatcaccca

SEQ ID NO: 56 - DNA, 36 bp, synthetic construct
  source 1..36: mol_type = other DNA
atgcctgcaggtcgacccttcattttaagttccttg

SEQ ID NO: 57 - DNA, 33 bp, synthetic construct
  source 1..33: mol_type = other DNA
cggtacccggggatccttcatcgatagggtggg

SEQ ID NO: 58 - DNA, 34 bp, synthetic construct
  source 1..34: mol_type = other DNA
gtactcctcagcttactcatcctttgcatcaaca

SEQ ID NO: 59 - DNA, 34 bp, synthetic construct
  source 1..34: mol_type = other DNA
agtaagctgaggagtactgcctgccaaccatcaa

SEQ ID NO: 60 - DNA, 34 bp, synthetic construct
  source 1..34: mol_type = other DNA
atgcctgcaggtcgaccgactggcttgccaccct

SEQ ID NO: 61 - DNA, 35 bp, synthetic construct
  source 1..35: mol_type = other DNA
cggtacccggggatcctgaccccaggcaagcacgg

SEQ ID NO: 62 - DNA, 27 bp, synthetic construct
  source 1..27: mol_type = other DNA
gaagcgagtacgagtttaagtcttatc

SEQ ID NO: 63 - DNA, 20 bp, synthetic construct
  source 1..20: mol_type = other DNA
aaactcgtactcgcttctcc

SEQ ID NO: 64 - DNA, 35 bp, synthetic construct
  source 1..35: mol_type = other DNA
atgcctgcaggtcgaccggcgccggcaacctcgtc